European Patent Application EP 4 506 018 A1, published February 12, 2025. Title: A novel anticancer agent targeting tumor antigen. Applicant: INDUSTRY FOUNDATION OF CHONNAM NATIONAL UNIVERSITY. Application KR PD23-6295, filed April 5, 2023. The sequence listing filed with the application follows.

SEQUENCE LISTING (35 sequences)

SEQ ID NO: 1 - DNA, 318 bp, synthetic construct
  misc_feature 1..318: note = CRT1
  source 1..318: mol_type = other DNA
atggctagcgtttctgatgttccgagggacctggaagttgttgctgcgacccccaccagcctactgatcagctgggatgctcctgctgtcacagtgagatattacaggatcacttacggagaaacaggaggaaatagccctgtccaggagttcactgtgcctgggagcaagtctacagctaccatcagcggccttaaacctggagttgattataccatcactgtgtatgctgtcactggtcaaccaatgtatggtcaaccaatgtatccaatttccattaattaccgaacaggatcccaccatcaccatcatcactga

SEQ ID NO: 2 - DNA, 309 bp, synthetic construct
  misc_feature 1..309: note = CRT2
  source 1..309: mol_type = other DNA
atggctagcgtttctgatgttccgagggacctggaagttgttgctgcgacccccaccagcctactgatcagctgggatgctcctgctgtcacagtgagatattacaggatcacttacggagaaacaggaggaaatagccctgtccaggagttcactgtgcctgggagcaagtctacagctaccatcagcggccttaaacctggagttgattataccatcactgtgtatgctgtcactaaattaggtttttttaaaagaccaatttccattaattaccgaacaggatcccaccatcaccatcatcactga

SEQ ID NO: 3 - DNA, 315 bp, synthetic construct
  misc_feature 1..315: note = CRT3
  source 1..315: mol_type = other DNA
atggctagcgtttctgatgttccgagggacctggaagttgttgctgcgacccccaccagcctactgatcagctggaaattaggtttttttaaaagatattacaggatcacttacggagaaacaggaggaaatagccctgtccaggagttcactgtgcctgggagcaagtctacagctaccatcagcggccttaaacctggagttgattataccatcactgtgtatgctgtcactggtcaaccaatgtatggtcaaccaatgtatccaatttccattaattaccgaacaggatcccaccatcaccatcatcactga

SEQ ID NO: 4 - DNA, 315 bp, synthetic construct
  misc_feature 1..315: note = CRT4
  source 1..315: mol_type = other DNA
atggctagcgtttctgatgttccgagggacctggaagttgttgctgcgacccccaccagcctactgatcagctggggtcaaccaatgtatggtcaaccaatgtattattacaggatcacttacggagaaacaggaggaaatagccctgtccaggagttcactgtgcctgggagcaagtctacagctaccatcagcggccttaaacctggagttgattataccatcactgtgtatgctgtcactaaattaggtttttttaaaagaccaatttccattaattaccgaacaggatcccaccatcaccatcatcactga

SEQ ID NO: 5 - DNA, 324 bp, synthetic construct
  misc_feature 1..324: note = CRT5
  source 1..324: mol_type = other DNA
atggctagcgtttctgatgttccgagggacctggaagttgttgctgcgacccccaccagcctactgatcagctggggtcaaccaatgtatggtcaaccaatgtattattacaggatcacttacggagaaacaggaggaaatagccctgtccaggagttcactgtgcctgggagcaagtctacagctaccatcagcggccttaaacctggagttgattataccatcactgtgtatgctgtcactggccgtggagacagccccgcaagcagcaagccaatttccattaattaccgaacaggatcccaccatcaccatcatcactga

SEQ ID NO: 6 - DNA, 315 bp, synthetic construct
  misc_feature 1..315: note = CRT6
  source 1..315: mol_type = other DNA
atggctagcgtttctgatgttccgagggacctggaagttgttgctgcgacccccaccagcctactgatcagctggaaattaggtttttttaaaagatattacaggatcacttacggagaaacaggaggaaatagccctgtccaggagttcactgtgcctgggagcaagtctacagctaccatcagcggccttaaacctggagttgattataccatcactgtgtatgctgtcactggccgtggagacagccccgcaagcagcaagccaatttccattaattaccgaacaggatcccaccatcaccatcatcactga

SEQ ID NO: 7 - protein, 105 aa, synthetic construct
  REGION 1..105: note = CRT1
MASVSDVPRDLEVVAATPTSLLISWDAPAVTVRYYRITYGETGGNSPVQEFTVPGSKSTATISGLKPGVDYTITVYAVTGQPMYGQPMYPISINYRTGSHHHHHH

SEQ ID NO: 8 - protein, 102 aa, synthetic construct
  REGION 1..102: note = CRT2
MASVSDVPRDLEVVAATPTSLLISWDAPAVTVRYYRITYGETGGNSPVQEFTVPGSKSTATISGLKPGVDYTITVYAVTKLGFFKRPISINYRTGSHHHHHH

SEQ ID NO: 9 - protein, 104 aa, synthetic construct
  REGION 1..104: note = CRT3
MASVSDVPRDLEVVAATPTSLLISWKLGFFKRYYRITYGETGGNSPVQEFTVPGSKSTATISGLKPGVDYTITVYAVTGQPMYGQPMYPISINYRTGSHHHHHH

SEQ ID NO: 10 - protein, 104 aa, synthetic construct
  REGION 1..104: note = CRT4
MASVSDVPRDLEVVAATPTSLLISWGQPMYGQPMYYYRITYGETGGNSPVQEFTVPGSKSTATISGLKPGVDYTITVYAVTKLGFFKRPISINYRTGSHHHHHH

SEQ ID NO: 11 - protein, 107 aa, synthetic construct
  REGION 1..107: note = CRT5
MASVSDVPRDLEVVAATPTSLLISWGQPMYGQPMYYYRITYGETGGNSPVQEFTVPGSKSTATISGLKPGVDYTITVYAVTGRGDSPASSKPISINYRTGSHHHHHH

SEQ ID NO: 12 - protein, 104 aa, synthetic construct
  REGION 1..104: note = CRT6
MASVSDVPRDLEVVAATPTSLLISWKLGFFKRYYRITYGETGGNSPVQEFTVPGSKSTATISGLKPGVDYTITVYAVTGRGDSPASSKPISINYRTGSHHHHHH

SEQ ID NO: 13 - DNA, 318 bp, synthetic construct
  misc_feature 1..318: note = DGR Scrambled monobody
  source 1..318: mol_type = other DNA
atggctagcgtttctgatgttccgagggacctggaagttgttgctgcgacccccaccagcctactgatcagctgggatgctcctgctgtcacagtgagatattacaggatcacttacggagaaacaggaggaaatagccctgtccaggagttcactgtgcctgggagcaagtctacagctaccatcagcggccttaaacctggagttgattataccatcactgtgtatgctgtcactggcgacggacgtagccccgcaagcagcaagccaatttccattaattaccgaacaggatcccaccatcaccatcatcactga

SEQ ID NO: 14 - protein, 105 aa, synthetic construct
  REGION 1..105: note = DGR Scrambled monobody
MASVSDVPRDLEVVAATPTSLLISWDAPAVTVRYYRITYGETGGNSPVQEFTVPGSKSTATISGLKPGVDYTITVYAVTGDGRSPASSKPISINYRTGSHHHHHH

SEQ ID NO: 15 - protein, 7 aa, synthetic construct
  REGION 1..7: note = Int-alpha
KLGFFKR

SEQ ID NO: 16 - protein, 10 aa, synthetic construct
  REGION 1..10: note = Hep-I
GQPMYGQPMY

SEQ ID NO: 17 - DNA, 31 bp, synthetic construct
  misc_feature 1..31: note = Nhe1
  source 1..31: mol_type = other DNA
tacatatggctagcgtttctgatgttccgag

SEQ ID NO: 18 - DNA, 38 bp, synthetic construct
  misc_feature 1..38: note = BamH1
  source 1..38: mol_type = other DNA
tactgagtggatcctgttcggtaattaatggaaattgg

SEQ ID NO: 19 - protein, 6 aa, synthetic construct
  REGION 1..6: note = tetracystein motif
CCXXCC

SEQ ID NO: 20 - protein, 326 aa, synthetic construct
  REGION 1..326: note = L-asparaginase
LPNITILATGGTIAGGGDSATKSNYTAGKVGVENLVNAVPQLKDIANVKGEQVVNIGSQDMNDDVWLTLAKKINTDCDKTDGFVITHGTDTMEETAYFLDLTVKCDKPVVMVGAMRPSTSMSADGPFNLYNAVVTAADKASANRGVLVVMNDTVLDGRDVTKTNTTDVATFKSVNYGPLGYIHNGKIDYQRTPARKHTSDTPFDVSKLNELPKVGIVYNYANASDLPAKALVDAGYDGIVSAGVGNGNLYKTVFDTLATAAKNGTAVVRSSRVPTGATTQDVEVDDAKYGFVASGTLNPQKARVLLQLALTQTKDPQQIQQIFNQY

SEQ ID NO: 21 - protein, 20 aa, synthetic construct
  REGION 1..20: note = PAS200 repeat unit
ASPAAPAPASPAAPAPSAPA

SEQ ID NO: 22 - protein, 201 aa, synthetic construct
  REGION 1..201: note = PAS200
ASPAAPAPASPAAPAPSAPAASPAAPAPASPAAPAPSAPAASPAAPAPASPAAPAPSAPAASPAAPAPASPAAPAPSAPAASPAAPAPASPAAPAPSAPAASPAAPAPASPAAPAPSAPAASPAAPAPASPAAPAPSAPAASPAAPAPASPAAPAPSAPAASPAAPAPASPAAPAPSAPAASPAAPAPASPAAPAPSAPAA

SEQ ID NO: 23 - protein, 656 aa, synthetic construct
  REGION 1..656: note = CRT3-Lasp-PAS200
MASVSDVPRDLEVVAATPTSLLISWKLGFFKRYYRITYGETGGNSPVQEFTVPGSKSTATISGLKPGVDYTITVYAVTGQPMYGQPMYPISINYRTSGGGGSGGGGSEFLPNITILATGGTIAGGGDSATKSNYTAGKVGVENLVNAVPQLKDIANVKGEQVVNIGSQDMNDDVWLTLAKKINTDCDKTDGFVITHGTDTMEETAYFLDLTVKCDKPVVMVGAMRPSTSMSADGPFNLYNAVVTAADKASANRGVLVVMNDTVLDGRDVTKTNTTDVATFKSVNYGPLGYIHNGKIDYQRTPARKHTSDTPFDVSKLNELPKVGIVYNYANASDLPAKALVDAGYDGIVSAGVGNGNLYKTVFDTLATAAKNGTAVVRSSRVPTGATTQDVEVDDAKYGFVASGTLNPQKARVLLQLALTQTKDPQQIQQIFNQYGSSGGGGSGGGGSASPAAPAPASPAAPAPSAPAASPAAPAPASPAAPAPSAPAASPAAPAPASPAAPAPSAPAASPAAPAPASPAAPAPSAPAASPAAPAPASPAAPAPSAPAASPAAPAPASPAAPAPSAPAASPAAPAPASPAAPAPSAPAASPAAPAPASPAAPAPSAPAASPAAPAPASPAAPAPSAPAASPAAPAPASPAAPAPSAPAAGSHHHHH

SEQ ID NO: 24 - protein, 657 aa, synthetic construct
  REGION 1..657: note = CRT4-Lasp-PAS200
MASVSDVPRDLEVVAATPTSLLISWGQPMYGQPMYYYRITYGETGGNSPVQEFTVPGSKSTATISGLKPGVDYTITVYAVTKLGFFKRPISINYRTSGGGGSGGGGSEFLPNITILATGGTIAGGGDSATKSNYTAGKVGVENLVNAVPQLKDIANVKGEQVVNIGSQDMNDDVWLTLAKKINTDCDKTDGFVITHGTDTMEETAYFLDLTVKCDKPVVMVGAMRPSTSMSADGPFNLYNAVVTAADKASANRGVLVVMNDTVLDGRDVTKTNTTDVATFKSVNYGPLGYIHNGKIDYQRTPARKHTSDTPFDVSKLNELPKVGIVYNYANASDLPAKALVDAGYDGIVSAGVGNGNLYKTVFDTLATAAKNGTAVVRSSRVPTGATTQDVEVDDAKYGFVASGTLNPQKARVLLQLALTQTKDPQQIQQIFNQYGSSGGGGSGGGGSASPAAPAPASPAAPAPSAPAASPAAPAPASPAAPAPSAPAASPAAPAPASPAAPAPSAPAASPAAPAPASPAAPAPSAPAASPAAPAPASPAAPAPSAPAASPAAPAPASPAAPAPSAPAASPAAPAPASPAAPAPSAPAASPAAPAPASPAAPAPSAPAASPAAPAPASPAAPAPSAPAASPAAPAPASPAAPAPSAPAAGSHHHHHH

SEQ ID NO: 25 - DNA, 1974 bp, synthetic construct
  misc_feature 1..1974: note = polynucleotide encoding CRT3-Lasp-PAS200
  source 1..1974: mol_type = other DNA
atggctagcgtttctgatgttccgagggacctggaagttgttgctgcgacccccaccagcctactgatcagctggaaattaggtttttttaaaagatattacaggatcacttacggagaaacaggaggaaatagccctgtccaggagttcactgtgcctgggagcaagtctacagctaccatcagcggccttaaacctggagttgattataccatcactgtgtatgctgtcactggtcaaccaatgtatggtcaaccaatgtatccaatttccattaattaccgaacaagcggcggcggcggcagcggcggcggcggcagcgaattcttacccaatatcaccattttagcaaccggcgggaccattgccggtggtggtgactccgcaaccaaatctaactacacagcgggtaaagttggcgtagaaaatctggttaatgcggtgccgcaactgaaggacattgcgaacgttaaaggcgagcaggtagtgaatattggctcccaggacatgaacgatgatgtctggctgacactggcgaaaaaaattaacaccgactgcgataagaccgacggcttcgtcattacccacggtaccgacacgatggaagaaactgcttacttcctcgacctgacggtgaaatgcgacaaaccggtggtgatggtcggtgcaatgcgtccgtccacgtctatgagcgcagacggtccattcaacctgtataacgcggtagtgactgcagctgataaagcctccgctaatcgtggcgtactggtagtgatgaacgacaccgtgcttgatggccgtgatgtcaccaaaaccaacaccaccgatgtagcgaccttcaagtctgttaactacggtcctctgggttacattcacaacggtaagattgactaccaacgtaccccggcacgtaagcacaccagcgacacgccgttcgatgtctctaagctgaatgaactgccgaaagtcggcattgtttataactacgctaacgcatccgatcttccggctaaagcactggtagatgcgggctatgatggcatcgttagcgctggcgtgggtaacggcaacctgtataaaaccgtatttgacacccttgcaaccgctgcgaaaaacggcactgcagtagtgcgttcttcccgcgtaccgacgggcgctaccactcaggatgtcgaagtggatgatgcgaaatacggcttcgtcgcctctggcacgttgaacccgcaaaaagcgcgcgttctgctgcaactggctctgacgcaaactaaagatccgcagcagatccagcagatcttcaatcagtacggatctagcggcggcggcggcagcggcggcggcggcagcgctagtccagccgctccagcacctgcatctccagcagctcccgctcctagtgcacccgctgcttcgcctgctgctccggctcctgcttcccccgctgcaccggcaccttcagctccagcagcatccccagcagcgccagctccagcgtccccagctgcaccagcacctagcgctcctgctgcaagccctgctgcaccagcgcctgcctctcctgcggctcctgctccatcggcgccagcagcttcgccagcagcacctgcccctgcaagcccagcagcaccggcaccttctgcacctgcagctagtccagccgctccagcacctgcatctccagcagctcccgctcctagtgcacccgctgcttcgcctgctgctccggctcctgcttcccccgctgcaccggcaccttcagctccagcagcatccccagcagcgccagctccagcgtccccagctgcaccagcacctagcgctcctgctgcaagcccagctgcaccagcgcctgcctctcctgcggctcctgctccatcggcgccagcagcttcgccagcagcacctgcccctgcaagcccagcagcaccggcaccttctgcacctgccgcaggatcccaccatcaccatcatcactga

SEQ ID NO: 26 - DNA, 1974 bp, synthetic construct
  misc_feature 1..1974: note = polynucleotide encoding CRT4-Lasp-PAS200
  source 1..1974: mol_type = other DNA
atggctagcgtttctgatgttccgagggacctggaagttgttgctgcgacccccaccagcctactgatcagctggggtcaaccaatgtatggtcaaccaatgtattattacaggatcacttacggagaaacaggaggaaatagccctgtccaggagttcactgtgcctgggagcaagtctacagctaccatcagcggccttaaacctggagttgattataccatcactgtgtatgctgtcactaaattaggtttttttaaaagaccaatttccattaattaccgaacaagcggcggcggcggcagcggcggcggcggcagcgaattcttacccaatatcaccattttagcaaccggcgggaccattgccggtggtggtgactccgcaaccaaatctaactacacagcgggtaaagttggcgtagaaaatctggttaatgcggtgccgcaactgaaggacattgcgaacgttaaaggcgagcaggtagtgaatattggctcccaggacatgaacgatgatgtctggctgacactggcgaaaaaaattaacaccgactgcgataagaccgacggcttcgtcattacccacggtaccgacacgatggaagaaactgcttacttcctcgacctgacggtgaaatgcgacaaaccggtggtgatggtcggtgcaatgcgtccgtccacgtctatgagcgcagacggtccattcaacctgtataacgcggtagtgactgcagctgataaagcctccgctaatcgtggcgtactggtagtgatgaacgacaccgtgcttgatggccgtgatgtcaccaaaaccaacaccaccgatgtagcgaccttcaagtctgttaactacggtcctctgggttacattcacaacggtaagattgactaccaacgtaccccggcacgtaagcacaccagcgacacgccgttcgatgtctctaagctgaatgaactgccgaaagtcggcattgtttataactacgctaacgcatccgatcttccggctaaagcactggtagatgcgggctatgatggcatcgttagcgctggcgtgggtaacggcaacctgtataaaaccgtatttgacacccttgcaaccgctgcgaaaaacggcactgcagtagtgcgttcttcccgcgtaccgacgggcgctaccactcaggatgtcgaagtggatgatgcgaaatacggcttcgtcgcctctggcacgttgaacccgcaaaaagcgcgcgttctgctgcaactggctctgacgcaaactaaagatccgcagcagatccagcagatcttcaatcagtacggatctagcggcggcggcggcagcggcggcggcggcagcgctagtccagccgctccagcacctgcatctccagcagctcccgctcctagtgcacccgctgcttcgcctgctgctccggctcctgcttcccccgctgcaccggcaccttcagctccagcagcatccccagcagcgccagctccagcgtccccagctgcaccagcacctagcgctcctgctgcaagccctgctgcaccagcgcctgcctctcctgcggctcctgctccatcggcgccagcagcttcgccagcagcacctgcccctgcaagcccagcagcaccggcaccttctgcacctgcagctagtccagccgctccagcacctgcatctccagcagctcccgctcctagtgcacccgctgcttcgcctgctgctccggctcctgcttcccccgctgcaccggcaccttcagctccagcagcatccccagcagcgccagctccagcgtccccagctgcaccagcacctagcgctcctgctgcaagcccagctgcaccagcgcctgcctctcctgcggctcctgctccatcggcgccagcagcttcgccagcagcacctgcccctgcaagcccagcagcaccggcaccttctgcacctgccgcaggatcccaccatcaccatcatcactga

SEQ ID NO: 27 - protein, 90 aa, synthetic construct
  REGION 1..90: note = Monobody specific for human EphA2 EM1
VSDVPRDLEVVAATPTSLLISWYYPFCAFYYRITYGETGGNSPVQEFTVPRSPDTATISGLKPGVDYTITVYAVTCLGSYSRPISINYRT

SEQ ID NO: 28 - protein, 652 aa, synthetic construct
  REGION 1..652: note = EM1-L-asp-PAS200
MVSDVPRDLEVVAATPTSLLISWYYPFCAFYYRITYGETGGNSPVQEFTVPRSPDTATISGLKPGVDYTITVYAVTCLGSYSRPISINYRTSGGGGSGGGGSEFLPNITILATGGTIAGGGDSATKSNYTAGKVGVENLVNAVPQLKDIANVKGEQVVNIGSQDMNDDVWLTLAKKINTDCDKTDGFVITHGTDTMEETAYFLDLTVKCDKPVVMVGAMRPSTSMSADGPFNLYNAVVTAADKASANRGVLVVMNDTVLDGRDVTKTNTTDVATFKSVNYGPLGYIHNGKIDYQRTPARKHTSDTPFDVSKLNELPKVGIVYNYANASDLPAKALVDAGYDGIVSAGVGNGNLYKTVFDTLATAAKNGTAVVRSSRVPTGATTQDVEVDDAKYGFVASGTLNPQKARVLLQLALTQTKDPQQIQQIFNQYGSSGGGGSGGGGSASPAAPAPASPAAPAPSAPAASPAAPAPASPAAPAPSAPAASPAAPAPASPAAPAPSAPAASPAAPAPASPAAPAPSAPAASPAAPAPASPAAPAPSAPAASPAAPAPASPAAPAPSAPAASPAAPAPASPAAPAPSAPAASPAAPAPASPAAPAPSAPAASPAAPAPASPAAPAPSAPAASPAAPAPASPAAPAPSAPAAGSHHHHHH

SEQ ID NO: 29 - DNA, 1989 bp, synthetic construct
  misc_feature 1..1989: note = polynucleotide encoding EM1-L-asp-PAS200
  source 1..1989: mol_type = other DNA
atggtgagcgatgtgccgcgcgatctggaagtggtggcggcgaccccgaccagcctgctgattagctggtattatccgttttgcgcgttttattatcgcattacctatggcgaaaccggcggcaacagcccggtgcaggaatttaccgtgccgcgcagcccggataccgcgaccattagcggcctgaaaccgggcgtggattataccattaccgtgtatgcggtgacctgcctgggcagctatagccgcccgattagcattaactatcgcaccaaaagaccaatttccattaattaccgaacaagcggcggcggcggcagcggcggcggcggcagcgaattcttacccaatatcaccattttagcaaccggcgggaccattgccggtggtggtgactccgcaaccaaatctaactacacagcgggtaaagttggcgtagaaaatctggttaatgcggtgccgcaactgaaggacattgcgaacgttaaaggcgagcaggtagtgaatattggctcccaggacatgaacgatgatgtctggctgacactggcgaaaaaaattaacaccgactgcgataagaccgacggcttcgtcattacccacggtaccgacacgatggaagaaactgcttacttcctcgacctgacggtgaaatgcgacaaaccggtggtgatggtcggtgcaatgcgtccgtccacgtctatgagcgcagacggtccattcaacctgtataacgcggtagtgactgcagctgataaagcctccgctaatcgtggcgtactggtagtgatgaacgacaccgtgcttgatggccgtgatgtcaccaaaaccaacaccaccgatgtagcgaccttcaagtctgttaactacggtcctctgggttacattcacaacggtaagattgactaccaacgtaccccggcacgtaagcacaccagcgacacgccgttcgatgtctctaagctgaatgaactgccgaaagtcggcattgtttataactacgctaacgcatccgatcttccggctaaagcactggtagatgcgggctatgatggcatcgttagcgctggcgtgggtaacggcaacctgtataaaaccgtatttgacacccttgcaaccgctgcgaaaaacggcactgcagtagtgcgttcttcccgcgtaccgacgggcgctaccactcaggatgtcgaagtggatgatgcgaaatacggcttcgtcgcctctggcacgttgaacccgcaaaaagcgcgcgttctgctgcaactggctctgacgcaaactaaagatccgcagcagatccagcagatcttcaatcagtacggatctagcggcggcggcggcagcggcggcggcggcagcgctagtccagccgctccagcacctgcatctccagcagctcccgctcctagtgcacccgctgcttcgcctgctgctccggctcctgcttcccccgctgcaccggcaccttcagctccagcagcatccccagcagcgccagctccagcgtccccagctgcaccagcacctagcgctcctgctgcaagccctgctgcaccagcgcctgcctctcctgcggctcctgctccatcggcgccagcagcttcgccagcagcacctgcccctgcaagcccagcagcaccggcaccttctgcacctgcagctagtccagccgctccagcacctgcatctccagcagctcccgctcctagtgcacccgctgcttcgcctgctgctccggctcctgcttcccccgctgcaccggcaccttcagctccagcagcatccccagcagcgccagctccagcgtccccagctgcaccagcacctagcgctcctgctgcaagcccagctgcaccagcgcctgcctctcctgcggctcctgctccatcggcgccagcagcttcgccagcagcacctgcccctgcaagcccagcagcaccggcaccttctgcacctgccgcaggatcccaccatcaccatcatcactga

SEQ ID NO: 30 - DNA, 68 bp, synthetic construct
  misc_feature 1..68: note = BglII-G4S-PAS200-F
  source 1..68: mol_type = other DNA
acaagatctagcggcggcggcggcagcggcggcggcggcagcgctagtccagccgctccagcacctgc

SEQ ID NO: 31 - DNA, 25 bp, synthetic construct
  misc_feature 1..25: note = pET-R
  source 1..25: mol_type = other DNA
ttattgctcagcggtggcagcagcc

SEQ ID NO: 32 - DNA, 34 bp, synthetic construct
  misc_feature 1..34: note = LASP-EcoR1-F
  source 1..34: mol_type = other DNA
ggcagcgaattcttacccaatatcaccattttag

SEQ ID NO: 33 - DNA, 36 bp, synthetic construct
  misc_feature 1..36: note = LASP-BamH1-R
  source 1..36: mol_type = other DNA
gccgctggatccgtactgattgaagatctgctggat

SEQ ID NO: 34 - DNA, 26 bp, synthetic construct
  misc_feature 1..26: note = T7
  source 1..26: mol_type = other DNA
taatacgactcactataggggaattg

SEQ ID NO: 35 - DNA, 81 bp, synthetic construct
  misc_feature 1..81: note = 94old(GC)-R
  source 1..81: mol_type = other DNA
caggccctgcagaagcttgaattcgctgccgccgccgccgctgccgccgccgccgcttgttcggtaattaatggaaattgg